European Patent Application EP 4 361 274 A1, published May 1, 2024. Title: Laccase. Applicant: Amano Enzyme Inc. The sequence listing filed with the application follows.

SEQUENCE LISTING (3 sequences)

SEQ ID NO: 1 - protein, 587 aa, Paramyrothecium sp.
MVARNLGLLALNLGLLKEVAALPKTGLLKRQTQAQISPEIGVYEEPLPIPPVKQPKHIIENPITGADIQYYEINIQPFTHSVYPDLDATELTGYDGISPGPTIIVPRNTETVVRFVNNAAQENSVHLHGSYSRAPFDGWAEDVTNPGEYKDYYYPNQQSGRLLWYHDHAMHITAENAYRGQAGAYILTDPAEDALNLPSGYGVHDIPLILTSKQYNQDGTLWDFAAATGAWYGDVIHVNGQPWPFFNVEPRKYRFRILNAAVSRSFALYFADSTDTSEELPFQVIASDSGLLTGPVETDHLFISMAERYEVVFDFSQYAGQTIDLRNQDSAGGVGTDANFENTDKVLRFQVASELSEPDTSEVPTTLRNVPFPEGGEGIDHVFDFERVNNQWTINGVTFADVENRILAEVPRDTVEIWELSNDSNFWSHPIHVHLVDFKILSRSNGRLEEYESAGLKDVVWLGKGETALVEAHYAPWPGVYMFHCHNLIHEDDDMMAAFNVTVLPNYGYNETTYLDPMEEEWRAKPFDASDFTAQSGPFSLNTITERIEFMASFQPYLDDSTVDPNSPEATAAGRRAKRGNITVRRK

SEQ ID NO: 2 - DNA, 1764 bp, Paramyrothecium sp.
atggtcgctcgtaacctcgggcttttggctctcaacttgggcctcctcaaggaggtcgccgctcttcccaagacaggattgctcaagagacagactcaggcgcagattagtcctgaaattggcgtctacgaagagcctctgccaatccctcctgtcaagcagcccaagcacatcattgaaaaccccatcactggagcagatatccagtactatgagatcaatattcagccattcacccattctgtttaccctgatcttgatgctacggagctcaccggctatgatggcatctctcctgggccaaccatcatcgtcccgcgtaacaccgagacggtggtgcgcttcgtcaataatgcagctcaggagaactccgtgcatctgcacggttcgtactcccgtgctccatttgatggatgggccgaggatgtgaccaaccccggggagtataaggattattactaccctaaccagcagagcggccgtctcctgtggtaccatgaccatgctatgcatattactgccgaaaacgcctacagaggccaggctggtgcatacattctcacagaccctgctgaggatgcacttaacctgccgagtggctatggtgtgcacgacattccgcttatccttacgtcgaagcagtacaaccaggatggaactctctgggactttgctgccgccaccggcgcctggtatggcgatgtcatccatgtgaatggacaaccttggccctttttcaatgtcgagccccgcaagtaccgcttccgcatcttgaatgctgctgtctctcgatcattcgctctttactttgccgactctacggacacctctgaggagctacctttccaagttattgcttcagattctggccttttgactggcccagtcgagactgaccacttgttcatctctatggctgagcgttacgaagtcgtttttgatttctcccagtacgcgggtcagacgatcgatctccgaaaccaagatagtgcgggcggtgtgggcacggatgccaactttgagaacaccgacaaggtcctgcgattccaagttgcttctgagctctctgagccggatacctcagaggtccctactaccctccgcaacgttcccttccctgaaggaggcgagggtatcgatcacgtctttgacttcgaacgcgtcaacaaccagtggactatcaacggcgtgacttttgccgatgttgagaaccgcattcttgctgaagtcccacgtgacaccgtcgagatctgggagctttcgaacgattctaacttctggtcccaccccattcacgtccacctcgttgactttaagatcttgtctcgatccaacggtcgacttgaggagtatgagtctgctggtctgaaggatgttgtctggctaggcaagggtgaaaccgctctggttgaggctcactacgctccctggcccggagtttacatgttccattgccacaacctaatccatgaagacgacgatatgatggctgcattcaatgtgaccgtccttcccaactacggctacaacgagaccacgtacctcgaccccatggaggaggagtggcgtgccaagcctttcgacgcttctgacttcacggcgcagtcaggcccattcagcctgaacacgatcaccgagcgtattgaattcatggcaagcttccagccatatcttgatgactctacggtggacccaaattctcctgaggctaccgctgctgggcgtcgtgccaagcgcggtaacattactgtccgccgtaagtaa

SEQ ID NO: 3 - DNA, 2018 bp, Paramyrothecium sp.
atggtcgctcgtaacctcgggcttttggctctcaacttgggcctcctcaaggaggtcgccgctcttcccaagacaggattgctcaagagacagactcaggcgcagattagtcctgaaattggcgtctacgaagagcctctgccaatccctcctgtcaagcagcccaagcagtaggcgttctctacagtttctactttaccctgcggctcacagttcttagcatcattgaaaaccccatcactggagcagatatccagtactatgagatcaatattcagccattcacccattctgtttaccctgatcttgatgctacggagctcaccggctatgatggcatctctcctgggccaaccatcatcgtcccgcgtaacaccgagacggtggtgcgcttcgtcaataatgcagctcaggagaactccgtgcatctgcacggttcgtactcccgtgctccatttgatggatgggccgaggatgtgaccaaccccggggagtataaggattattactaccctaaccagcagagcggccgtctcctgtggtaccatgaccatgctatgcatattgtaagtcaatcatcctggaggtcagaaaccccaactaattgcgacagactgccgaaaacgcctacagaggccaggctggtgcatacattctcacagaccctgctgaggatgcacttaacctgccgagtggctatggtgtgcacgacattccgcttatccttacgtcgaagcagtacaaccaggatggaactctctgggactttgctgccgccaccggcgcctggtatggcgatgtcatccatgtggtaagtcacttcgggcattggactatatatagaagctgacattgaacagaatggacaaccttggccctttttcaatgtcgagccccgcaagtaccgcttccgcatcttgaatgctgctgtctctcgatcattcgctctttactttgccgactctacggacacctctgaggagctacctttccaagttattgcttcagattctggccttttgactggcccagtcgagactgaccacttggtatatctccaatttccccaactcttcggcagaagctaactacagtttcagttcatctctatggctgagcgttacgaagtcgtttttgatttctcccagtacgcgggtcagacgatcgatctccgaaaccaagatagtgcgggcggtgtgggcacggatgccaactttgagaacaccgacaaggtcctgcgattccaagttgcttctgagctctctgagccggatacctcagaggtccctactaccctccgcaacgttcccttccctgaaggaggcgagggtatcgatcacgtctttgacttcgaacgcgtcaacaaccagtggactatcaacggcgtgacttttgccgatgttgagaaccgcattcttgctgaagtcccacgtgacaccgtcgagatctgggagctttcgaacgattctaacttctggtcccaccccattcacgtccacctcgttgactttaagatcttgtctcgatccaacggtcgacttgaggagtatgagtctgctggtctgaaggatgttgtctggctaggcaagggtgaaaccgctctggttgaggctcactacgctcccgtacgtacacacctttcctcatgtgcctctttgctctgtgctaacaatgcttcttagtggcccggagtttacatgttccattgccacaacctaatccatgaagacgacgatatgatggctgcattcaatgtgaccgtccttcccaactacggctacaacgagaccacgtacctcgaccccatggaggaggagtggcgtgccaagcctttcgacgcttctgacttcacggcgcagtcaggcccattcagcctgaacacgatcaccgagcgtattgaattcatggcaagcttccagccatatcttgatgactctacggtggacccaaattctcctgaggctaccgctgctgggcgtcgtgccaagcgcggtaacattactgtccgccgtaagtaa